European Patent Specification EP 2 998 740 B1, published July 5, 2023. Title: Methods for predicting clinical effects in immunotherapy. Applicant: International Institute of Cancer Immunology, Inc. Application PCT/JP2014/62630. The sequence listing filed with the application follows.

SEQUENCE LISTING (71 sequences)

SEQ ID NO: 1 - protein, 449 aa, Homo sapiens
MGSDVRDLNALLPAVPSLGGGGGCALPVSGAAQWAPVLDFAPPGASAYGSLGGPAPPPAPPPPPPPPPHSFIKQEPSWGGAEPHEEQCLSAFTVHFSGQFTGTAGACRYGPFGPPPPSQASSGQARMFPNAPYLPSCLESQPAIRNQGYSTVTFDGTPSYGHTPSHHAAQFPNHSFKHEDPMGQQGSLGEQQYSVPPPVYGCHTPTDSCTGSQALLLRTPYSSDNLYQMTSQLECMTWNQMNLGATLKGVAAGSSSSVKWTEGQSNHSTGYESDNHTTPILCGAQYRIHTHGVFRGIQDVRRVPGVAPTLVRSASETSEKRPFMCAYPGCNKRYFKLSHLQMHSRKHTGEKPYQCDFKDCERRFSRSDQLKRHQRRHTGVKPFQCKTCQRKFSRSDHLKTHTRTHTGKTSEKPFSCRWPSCQKKFARSDELVRHHNMHQRNMTKLQLAL

SEQ ID NO: 2 - protein, 9 aa, Artificial Sequence
  Synthetic polypeptide
CMTWNQMNL

SEQ ID NO: 3 - protein, 9 aa, Artificial Sequence
  Synthetic polypeptide
CYTWNQMNL

SEQ ID NO: 4 - protein, 9 aa, Artificial Sequence
  Synthetic polypeptide
RMFPNAPYL

SEQ ID NO: 5 - protein, 9 aa, Artificial Sequence
  Synthetic polypeptide
SLGEQQYSV

SEQ ID NO: 6 - protein, 16 aa, Artificial Sequence
  Synthetic polypeptide
KRYFKLSHLQMHSRKH

SEQ ID NO: 7 - protein, 18 aa, Artificial Sequence
  Synthetic polypeptide
MGSDVRDLNALLPAVPSL

SEQ ID NO: 8 - protein, 18 aa, Artificial Sequence
  Synthetic polypeptide
ALLPAVPSLGGGGGCALP

SEQ ID NO: 9 - protein, 18 aa, Artificial Sequence
  Synthetic polypeptide
GGGGGCALPVSGAAQWAP

SEQ ID NO: 10 - protein, 18 aa, Artificial Sequence
  Synthetic polypeptide
VSGAAQWAPVLDFAPPGA

SEQ ID NO: 11 - protein, 18 aa, Artificial Sequence
  Synthetic polypeptide
VLDFAPPGASAYGSLGGP

SEQ ID NO: 12 - protein, 18 aa, Artificial Sequence
  Synthetic polypeptide
SAYGSLGGPAPPPAPPPP

SEQ ID NO: 13 - protein, 18 aa, Artificial Sequence
  Synthetic polypeptide
APPPAPPPPPPPPPHSFI

SEQ ID NO: 14 - protein, 18 aa, Artificial Sequence
  Synthetic polypeptide
PPPPPHSFIKQEPSWGGA

SEQ ID NO: 15 - protein, 18 aa, Artificial Sequence
  Synthetic polypeptide
KQEPSWGGAEPHEEQCLS

SEQ ID NO: 16 - protein, 18 aa, Artificial Sequence
  Synthetic polypeptide
EPHEEQCLSAFTVHFSGQ

SEQ ID NO: 17 - protein, 18 aa, Artificial Sequence
  Synthetic polypeptide
AFTVHFSGQFTGTAGACR

SEQ ID NO: 18 - protein, 18 aa, Artificial Sequence
  Synthetic polypeptide
FTGTAGACRYGPFGPPPP

SEQ ID NO: 19 - protein, 18 aa, Artificial Sequence
  Synthetic polypeptide
YGPFGPPPPSQASSGQAR

SEQ ID NO: 20 - protein, 18 aa, Artificial Sequence
  Synthetic polypeptide
SQASSGQARMFPNAPYLP

SEQ ID NO: 21 - protein, 18 aa, Artificial Sequence
  Synthetic polypeptide
MFPNAPYLPSCLESQPAI

SEQ ID NO: 22 - protein, 18 aa, Artificial Sequence
  Synthetic polypeptide
SCLESQPAIRNQGYSTVT

SEQ ID NO: 23 - protein, 18 aa, Artificial Sequence
  Synthetic polypeptide
RNQGYSTVTFDGTPSYGH

SEQ ID NO: 24 - protein, 18 aa, Artificial Sequence
  Synthetic polypeptide
FDGTPSYGHTPSHHAAQF

SEQ ID NO: 25 - protein, 18 aa, Artificial Sequence
  Synthetic polypeptide
TPSHHAAQFPNHSFKHED

SEQ ID NO: 26 - protein, 18 aa, Artificial Sequence
  Synthetic polypeptide
PNHSFKHEDPMGQQGSLG

SEQ ID NO: 27 - protein, 18 aa, Artificial Sequence
  Synthetic polypeptide
PMGQQGSLGEQQYSVPPP

SEQ ID NO: 28 - protein, 18 aa, Artificial Sequence
  Synthetic polypeptide
VYGCHTPTDSCTGSQALL

SEQ ID NO: 29 - protein, 18 aa, Artificial Sequence
  Synthetic polypeptide
SCTGSQALLLRTPYSSDN

SEQ ID NO: 30 - protein, 18 aa, Artificial Sequence
  Synthetic polypeptide
LRTPYSSDNLYQMTSQLE

SEQ ID NO: 31 - protein, 18 aa, Artificial Sequence
  Synthetic polypeptide
LYQMTSQLECMTWNQMNL

SEQ ID NO: 32 - protein, 18 aa, Artificial Sequence
  Synthetic polypeptide
CMTWNQMNLGATLKGVAA

SEQ ID NO: 33 - protein, 18 aa, Artificial Sequence
  Synthetic polypeptide
GATLKGVAAGSSSSVKWT

SEQ ID NO: 34 - protein, 18 aa, Artificial Sequence
  Synthetic polypeptide
GSSSSVKWTEGQSNHSTG

SEQ ID NO: 35 - protein, 18 aa, Artificial Sequence
  Synthetic polypeptide
EGQSNHSTGYESDNHTTP

SEQ ID NO: 36 - protein, 18 aa, Artificial Sequence
  Synthetic polypeptide
YESDNHTTPILCGAQYRI

SEQ ID NO: 37 - protein, 18 aa, Artificial Sequence
  Synthetic polypeptide
ILCGAQYRIHTHGVFRGI

SEQ ID NO: 38 - protein, 18 aa, Artificial Sequence
  Synthetic polypeptide
HTHGVFRGIQDVRRVPGV

SEQ ID NO: 39 - protein, 18 aa, Artificial Sequence
  Synthetic polypeptide
QDVRRVPGVAPTLVRSAS

SEQ ID NO: 40 - protein, 18 aa, Artificial Sequence
  Synthetic polypeptide
APTLVRSASETSEKRPFM

SEQ ID NO: 41 - protein, 18 aa, Artificial Sequence
  Synthetic polypeptide
ETSEKRPFMCAYPGCNKR

SEQ ID NO: 42 - protein, 18 aa, Artificial Sequence
  Synthetic polypeptide
CAYPGCNKRYFKLSHLQM

SEQ ID NO: 43 - protein, 18 aa, Artificial Sequence
  Synthetic polypeptide
YFKLSHLQMHSRKHTGEK

SEQ ID NO: 44 - protein, 18 aa, Artificial Sequence
  Synthetic polypeptide
HSRKHTGEKPYQCDFKDC

SEQ ID NO: 45 - protein, 18 aa, Artificial Sequence
  Synthetic polypeptide
PYQCDFKDCERRFSRSDQ

SEQ ID NO: 46 - protein, 18 aa, Artificial Sequence
  Synthetic polypeptide
ERRFSRSDQLKRHQRRHT

SEQ ID NO: 47 - protein, 18 aa, Artificial Sequence
  Synthetic polypeptide
LKRHQRRHTGVKPFQCKT

SEQ ID NO: 48 - protein, 18 aa, Artificial Sequence
  Synthetic polypeptide
GVKPFQCKTCQRKFSRSD

SEQ ID NO: 49 - protein, 18 aa, Artificial Sequence
  Synthetic polypeptide
CQRKFSRSDHLKTHTRTH

SEQ ID NO: 50 - protein, 18 aa, Artificial Sequence
  Synthetic polypeptide
HLKTHTRTHTGKTSEKPF

SEQ ID NO: 51 - protein, 18 aa, Artificial Sequence
  Synthetic polypeptide
TGKTSEKPFSCRWPSCQK

SEQ ID NO: 52 - protein, 18 aa, Artificial Sequence
  Synthetic polypeptide
SCRWPSCQKKFARSDELV

SEQ ID NO: 53 - protein, 18 aa, Artificial Sequence
  Synthetic polypeptide
KFARSDELVRHHNMHQRN

SEQ ID NO: 54 - protein, 17 aa, Artificial Sequence
  Synthetic polypeptide
RHHNMHQRNMTKLQLAL

SEQ ID NO: 55 - protein, 18 aa, Artificial Sequence
  Synthetic polypeptide
MNLGATLKGHSTGYESDN

SEQ ID NO: 56 - protein, 18 aa, Artificial Sequence
  Synthetic polypeptide
KTHTRTHTGEKPFSCRWP

SEQ ID NO: 57 - protein, 132 aa, Artificial Sequence
  Synthetic polypeptide
SEKRPFMCAYPGCNKRYFKLSHLQMHSRKHTGEKPYQCDFKDCERRFSRSDQLKRHQRRHTGVKPFQCKTCQRKFSRSDHLKTHTRTHTGKTSEKPFSCRWPSCQKKFARSDELVRHHNMHQRNMTKLQLAL

SEQ ID NO: 58 - protein, 16 aa, Artificial Sequence
  Synthetic polypeptide
KRYFKLSHLQMHSRKH

SEQ ID NO: 59 - protein, 9 aa, Artificial Sequence
  Synthetic polypeptide
YFKLSHLQM

SEQ ID NO: 60 - protein, 7 aa, Artificial Sequence
  Synthetic polypeptide
KRYFKLS

SEQ ID NO: 61 - protein, 145 aa, Artificial Sequence
  Synthetic polypeptide
DPMGQQGSLGEQQYSVPPPVYGCHTPTDSCTGSQALLLRTPYSSDNLYQMTSQLECMTWNQMNLGATLKGVAAGSSSSVKWTEGQSNHSTGYESDNHTTPILCGAQYRIHTHGVFRGIQDVRRVPGVAPTLVRSASETSEKRPFM

SEQ ID NO: 62 - protein, 9 aa, Artificial Sequence
  Synthetic polypeptide
CMTWNQMNK

SEQ ID NO: 63 - protein, 7 aa, Artificial Sequence
  Synthetic polypeptide
TWNQMNL

SEQ ID NO: 64 - protein, 182 aa, Artificial Sequence
  Synthetic polypeptide
MGSDVRDLNALLPAVPSLGGGGGCALPVSGAAQWAPVLDFAPPGASAYGSLGGPAPPPAPPPPPPPPPHSFIKQEPSWGGAEPHEEQCLSAFTVHFSGQFTGTAGACRYGPFGPPPPSQASSGQARMFPNAPYLPSCLESQPAIRNQGYSTVTFDGTPSYGHTPSHHAAQFPNHSFKHEDPM

SEQ ID NO: 65 - protein, 9 aa, Artificial Sequence
  Synthetic polypeptide
RMFPNAPYL

SEQ ID NO: 66 - protein, 9 aa, Artificial Sequence
  Synthetic polypeptide
RMFPNAPYK

SEQ ID NO: 67 - protein, 7 aa, Artificial Sequence
  Synthetic polypeptide
FPNAPYL

SEQ ID NO: 68 - protein, 7 aa, Artificial Sequence
  Synthetic polypeptide
RMFPNAP

SEQ ID NO: 69 - protein, 6 aa, Artificial Sequence
  Synthetic polypeptide
PNAPYL

SEQ ID NO: 70 - protein, 6 aa, Artificial Sequence
  Synthetic polypeptide
RMFPNA

SEQ ID NO: 71 - protein, 5 aa, Artificial Sequence
  Synthetic polypeptide
RMFPN